European Patent Application EP 4 628 594 A1, published October 8, 2025. Title: METHODS OF AMPLIFYING DNA AND DNA PRODUCTS. Applicant: 4BASEBIO UK LTD. The sequence listing filed with the application follows.

SEQUENCE LISTING (3 sequences)

SEQ ID NO: 1 - DNA, 41 bp, synthetic construct
  source 1..41: mol_type = other DNA
agggctaacatttgttggccactcaggccaacaaatgttag

SEQ ID NO: 2 - DNA, 18 bp, synthetic construct
  source 1..18: mol_type = other DNA
  modified_base 14..18: mod_base = OTHER; note = nuclease resistant nucleotide
aaaaaaaaaaaaaaaaaa

SEQ ID NO: 3 - DNA, 14 bp, synthetic construct
  source 1..14: mol_type = other DNA
  modified_base 1..5: mod_base = OTHER; note = nuclease resistant nucleotide
tttttttttttttt